European Patent Application EP 4 714 973 A1, published March 25, 2026. Title: 特异性结合CLL1的抗体及其制法和应用. Applicant: 苏州亘喜生物科技有限公司. The sequence listing filed with the application follows.

SEQUENCE LISTING (59 sequences)

SEQ ID NO: 1 - protein, 113 aa, synthetic construct
QVQLVESGGGLVQPGGSLRLSCAASGFTFSSKTMGWARQVPGKAIEWLSGIYSDGSTYYADSVKGRFTISRDNAKNMVYLQMNSLKPEDTAVYYCATEDLTSYGRGTQVTVSS

SEQ ID NO: 2 - DNA, 339 bp, synthetic construct
  source 1..339: mol_type = other DNA
caagtgcaactggtggagtccggcgggggcctggtgcaacccggcggctccctgagactgagctgcgccgctagcggcttcaccttcagcagcaagaccatgggctgggctagacaagtgcccggcaaggccatcgagtggctgagcggcatctacagcgacggcagcacctactacgccgacagcgtgaagggcagattcaccatcagcagagacaacgccaagaacatggtgtacctgcagatgaacagcctgaagcccgaggacaccgccgtgtactactgcgccaccgaggacctgacaagctacggcagaggcacccaagtgaccgtgagcagc

SEQ ID NO: 3 - protein, 118 aa, synthetic construct
QVQLVESGGGLVQPGGSLRLSCAASGFTFSSYAMGWARQVPGKEVEWVSGIYSDGSTYYANSVKGRFTISRDNAKNTMYLQMNSLKPEDTAVYHCATDPTVHSDLPVWGQGTLVTVSS

SEQ ID NO: 4 - DNA, 354 bp, synthetic construct
  source 1..354: mol_type = other DNA
caagtgcaactcgtggagagcgggggggggctggtgcagcccggggggagcctgagactgagctgcgccgctagcggcttcaccttcagcagctacgccatgggctgggctagacaagtgcccggcaaagaggtggagtgggtgagcggcatctacagcgacggcagcacctactacgccaacagcgtgaagggcagattcaccatcagcagagacaacgccaagaacaccatgtacctgcagatgaacagcctgaagcccgaggacaccgccgtgtaccactgcgccacagatcccacagtgcacagcgatctgcccgtctgggggcaaggcaccctggtcaccgtgagcagc

SEQ ID NO: 5 - protein, 117 aa, synthetic construct
QVQLVESGGGLVQPGGSLRLSCAASGFTFSSYAMGWARQVPGKEVEWVSGIYSDGRTYYADSVKGRFTISRDNAKNEVYLQMNSLKPEDTAVYYCAPEPGQGVGDYWGQGTQVTVSS

SEQ ID NO: 6 - DNA, 351 bp, synthetic construct
  source 1..351: mol_type = other DNA
caagtgcagctcgtcgaaagcggcgggggcctggtgcaacctggcgggtccctgagactgagctgcgccgctagcggcttcaccttcagcagctacgccatgggctgggctagacaagtgcccggcaaagaggtggagtgggtgagcggcatctacagcgacggcagaacctactacgccgacagcgtgaagggcagattcaccatcagcagagacaacgccaagaacgaggtgtacctgcagatgaacagcctgaagcccgaggacaccgccgtctattactgtgcccccgagcctggccaaggcgtgggggattactggggccaaggcacccaagtgaccgtgagcagc

SEQ ID NO: 7 - protein, 118 aa, synthetic construct
QVQLVESGGGLVQPGGSLRLSCAASGFTFSSYAMGWARQVPGKDVEWVSGIYSDGSTNYADSVKGRFTISRDNAKNTVYLQMNSLRPEDTAVYHCATDPTVHSDLPVWGQGTLVTVSS

SEQ ID NO: 8 - DNA, 354 bp, synthetic construct
  source 1..354: mol_type = other DNA
caagtgcaactcgtggagagcgggggggggctggtgcagcccggggggagcctgagactgagctgcgccgctagcggcttcaccttcagcagctacgccatgggctgggctagacaagtgcccggcaaagacgtggagtgggtgagcggcatctacagcgacggcagcaccaactacgccgacagcgtgaagggcagattcaccatcagcagagacaacgccaagaacaccgtgtacctgcagatgaacagcctgagacccgaggacaccgccgtgtaccactgcgccacagatcccacagtgcacagcgatctgcccgtctgggggcaaggcaccctggtcaccgtgagcagc

SEQ ID NO: 9 - protein, 117 aa, synthetic construct
QVQLVESGGGLVQPGGSLRLSCAASGFTFSSYDMGWARQVPGKAVEWVSGIYSDGSTYYADSVKGRFTISRDNAKNTVYLQMNSLKPEDTAVYYCATDPLTSELRSWGQGTQVTVSS

SEQ ID NO: 10 - DNA, 351 bp, synthetic construct
  source 1..351: mol_type = other DNA
caagtgcagctggtcgaaagcggcggcgggctcgtgcagcccggcggcagcctgagactgagctgcgccgctagcggcttcaccttcagcagctacgacatgggctgggctagacaagtgcccggcaaggccgtggagtgggtgagcggcatctacagcgacggcagcacctactacgccgacagcgtgaagggcagattcaccatcagcagagacaacgccaagaacaccgtgtacctgcagatgaacagcctgaagcccgaggacaccgccgtgtactactgcgccaccgaccccctgacaagcgagctgagaagctggggccaaggcacccaagtgaccgtgagcagc

SEQ ID NO: 11 - protein, 118 aa, synthetic construct
QVQLVESGGGLVQPGGSLRLSCTASGFTFSSYAMGWARQVPGKEVEWVSGIYSDGSTNYADSVKGRFTISRDNAKNTVYLQMNSLRPEDTAVYHCATDPTVHSDLPVWGQGTLVTVSS

SEQ ID NO: 12 - DNA, 354 bp, synthetic construct
  source 1..354: mol_type = other DNA
caagtgcaactcgtggagagcgggggggggctggtgcagcccggggggagcctgagactgagctgcaccgctagcggcttcaccttcagcagctacgccatgggctgggctagacaagtgcccggcaaagaggtggagtgggtgagcggcatctacagcgacggcagcaccaactacgccgacagcgtgaagggcagattcaccatcagcagagacaacgccaagaacaccgtgtacctgcagatgaacagcctgagacccgaggacaccgccgtgtaccactgcgccacagatcccacagtgcacagcgatctgcccgtctgggggcaaggcaccctggtcaccgtgagcagc

SEQ ID NO: 13 - protein, 118 aa, synthetic construct
QVQLVESGGGLVQPGGSLRLSCAASGFTFSSYAMGWARQVPGKEVEWVSGIYSDGSTNYADSVKGRFTISRDNAKNTVYLQMNSLRPEDTAVYHCATDPTVHSDLPVWGQGTLVTVSS

SEQ ID NO: 14 - DNA, 354 bp, synthetic construct
  source 1..354: mol_type = other DNA
caagtgcaactcgtggagagcgggggggggctggtgcagcccggggggagcctgagactgagctgcgccgctagcggcttcaccttcagcagctacgccatgggctgggctagacaagtgcccggcaaagaggtggagtgggtgagcggcatctacagcgacggcagcaccaactacgccgacagcgtgaagggcagattcaccatcagcagagacaacgccaagaacaccgtgtacctgcagatgaacagcctgagacccgaggacaccgccgtgtaccactgcgccacagatcccacagtgcacagcgatctgcccgtctgggggcaaggcaccctggtcaccgtgagcagc

SEQ ID NO: 15 - protein, 118 aa, synthetic construct
QVQLVESGGGLVQPGGSLRLSCAASGFTFSSYAMGWARQVPGKEVEWVSGIYSDGSTNYADSVKGRFTISRDNAKNTVYLQMNSLRPEDTAVYHCATDPTVHSDLPVWGQGTQVTVSS

SEQ ID NO: 16 - DNA, 354 bp, synthetic construct
  source 1..354: mol_type = other DNA
caagtgcaactcgtggagagcgggggggggctggtgcagcccggggggagcctgagactgagctgcgccgctagcggcttcaccttcagcagctacgccatgggctgggctagacaagtgcccggcaaagaggtggagtgggtgagcggcatctacagcgacggcagcaccaactacgccgacagcgtgaagggcagattcaccatcagcagagacaacgccaagaacaccgtgtacctgcagatgaacagcctgagacccgaggacaccgccgtgtaccactgcgccacagatcccacagtgcacagcgatctgcccgtctgggggcaaggcacccaagtcaccgtgagcagc

SEQ ID NO: 17 - protein, 118 aa, synthetic construct
QVQLVESGGGLVQPGGSLRLSCAASGFTFSSYAMGWARQVPGKDVEWVSGIYSDGSTYYADSVKGRFTISRYNAKNTVYLQMNSLKPEDTAVYYCATDPTLENQTTAWGQGTQVTVSS

SEQ ID NO: 18 - DNA, 354 bp, synthetic construct
  source 1..354: mol_type = other DNA
caagtgcagctggtcgagagcggcgggggcctcgtccaacccggcggcagcctgagactgagctgcgccgctagcggcttcaccttcagcagctacgccatgggctgggctagacaagtgcccggcaaggacgtggagtgggtgagcggcatctacagcgacggcagcacctactacgccgacagcgtgaagggcagattcaccatcagcagatacaacgccaagaacaccgtgtacctgcagatgaacagcctgaagcccgaggacaccgccgtgtactactgcgccaccgatcctaccctcgagaatcagacaaccgcctggggccaagggacccaagtgaccgtgagcagc

SEQ ID NO: 19 - protein, 118 aa, synthetic construct
QVQLVESGGGLVQPGGSLRLACAASGFTFSSYAMGWARQVPGKDVEWVSGIYSDGSTYYADSVKGRFTISRDNAKNTVYLQMNSLKPEDTAVYYCATDPTLENQTTAWGQGTQVTVSS

SEQ ID NO: 20 - DNA, 354 bp, synthetic construct
  source 1..354: mol_type = other DNA
caagtgcaactggtcgaaagcgggggcggcctggtgcagcccggcggcagcctgagactggcctgcgccgctagcggcttcaccttcagcagctacgccatgggctgggctagacaagtgcccggcaaggacgtggagtgggtgagcggcatctacagcgacggcagcacctactacgccgacagcgtgaagggcagattcaccatcagcagagacaacgccaagaacaccgtgtacctgcagatgaacagcctgaagcccgaggacaccgccgtgtactactgcgccacagatcccacactggagaaccaaaccaccgcttgggggcaaggcacccaagtgaccgtgagcagc

SEQ ID NO: 21 - protein, 108 aa, synthetic construct
DIQMTQSPSSLSASLGERVSLTCRATQELSGYLSWLQQKPDGTIKRLIYAASTLDSGVPKRFSGNRSGSDYSLTISSLESEDFADYYCLQYAIYPYTFGGGTKLEIKR

SEQ ID NO: 22 - DNA, 324 bp, synthetic construct
  source 1..324: mol_type = other DNA
gacattcagatgacacagagccctagcagcctgagcgctagcctgggcgagagagtgagcctgacctgcagagccacccaagagctgagcggctacctgagctggctgcagcagaagcctgacggcaccatcaagagactgatctacgccgctagcaccctggacagcggcgtgcccaagagattcagcggcaacagaagcggcagcgactacagcctgaccatcagcagcctggagagcgaggacttcgccgactactactgcctgcagtacgccatctacccctacaccttcggcgggggcaccaagctggagatcaagaga

SEQ ID NO: 23 - protein, 120 aa, synthetic construct
EVQLQQSGPELVKPGASVKMSCKASGYTFTSYFIHWVKQKPGQGLEWIGFINPYNDGSKYNEKFKGKATLTSDKSSSTAYMELSSLTSEDSAVYYCTRDDGYYGYAMDYWGQGTSVTVSS

SEQ ID NO: 24 - DNA, 360 bp, synthetic construct
  source 1..360: mol_type = other DNA
gaggtgcagctgcagcagagcggccccgagctggtgaagcccggcgctagcgtgaagatgagctgcaaggctagcggctacaccttcacaagctacttcatccactgggtgaaacagaagcccggccaaggcctggagtggatcggcttcatcaacccctacaacgacggcagcaagtacaacgagaagttcaagggcaaggccaccctcacaagcgacaagagcagcagcaccgcctacatggagctgagcagcctgacaagcgaagacagcgccgtgtactactgcacaagagacgacggctactacggctacgccatggactactggggccaaggcacaagcgtcaccgtgagcagc

SEQ ID NO: 25 - protein, 15 aa, synthetic construct
GGGGSGGGGSGGGGS

SEQ ID NO: 26 - DNA, 45 bp, synthetic construct
  source 1..45: mol_type = other DNA
gggggcgggggcagcggcgggggggggagcggcgggggcggcagc

SEQ ID NO: 27 - protein, 243 aa, synthetic construct
EVQLQQSGPELVKPGASVKMSCKASGYTFTSYFIHWVKQKPGQGLEWIGFINPYNDGSKYNEKFKGKATLTSDKSSSTAYMELSSLTSEDSAVYYCTRDDGYYGYAMDYWGQGTSVTVSSGGGGSGGGGSGGGGSDIQMTQSPSSLSASLGERVSLTCRATQELSGYLSWLQQKPDGTIKRLIYAASTLDSGVPKRFSGNRSGSDYSLTISSLESEDFADYYCLQYAIYPYTFGGGTKLEIKR

SEQ ID NO: 28 - DNA, 729 bp, synthetic construct
  source 1..729: mol_type = other DNA
gaggtgcagctgcagcagagcggccccgagctggtgaagcccggcgctagcgtgaagatgagctgcaaggctagcggctacaccttcacaagctacttcatccactgggtgaaacagaagcccggccaaggcctggagtggatcggcttcatcaacccctacaacgacggcagcaagtacaacgagaagttcaagggcaaggccaccctcacaagcgacaagagcagcagcaccgcctacatggagctgagcagcctgacaagcgaagacagcgccgtgtactactgcacaagagacgacggctactacggctacgccatggactactggggccaaggcacaagcgtcaccgtgagcagcgggggcgggggcagcggcgggggggggagcggcgggggcggcagcgacattcagatgacacagagccctagcagcctgagcgctagcctgggcgagagagtgagcctgacctgcagagccacccaagagctgagcggctacctgagctggctgcagcagaagcctgacggcaccatcaagagactgatctacgccgctagcaccctggacagcggcgtgcccaagagattcagcggcaacagaagcggcagcgactacagcctgaccatcagcagcctggagagcgaggacttcgccgactactactgcctgcagtacgccatctacccctacaccttcggcgggggcaccaagctggagatcaagaga

SEQ ID NO: 29 - protein, 21 aa, synthetic construct
MALPVTALLLPLALLLHAARP

SEQ ID NO: 30 - DNA, 63 bp, synthetic construct
  source 1..63: mol_type = other DNA
atggccttaccagtgaccgccttgctcctgccgctggccttgctgctccacgccgccaggccg

SEQ ID NO: 31 - protein, 8 aa, synthetic construct
DYKDDDDK

SEQ ID NO: 32 - protein, 69 aa, synthetic construct
TTTPAPRPPTPAPTIASQPLSLRPEACRPAAGGAVHTRGLDFACDIYIWAPLAGTCGVLLLSLVITLYC

SEQ ID NO: 33 - DNA, 207 bp, synthetic construct
  source 1..207: mol_type = other DNA
acaacgacaccagcaccacggccacccactcctgctccgacaattgcgtctcagcccctttcccttcgacccgaagcttgtcgccctgctgcgggaggagcggtccacacgcgcgggcttgacttcgcttgcgacatctacatttgggcacccttggccgggacatgcggcgtcttgctcctgagtctggttataacgctgtattgt

SEQ ID NO: 34 - protein, 42 aa, synthetic construct
KRGRKKLLYIFKQPFMRPVQTTQEEDGCSCRFPEEEEGGCEL

SEQ ID NO: 35 - DNA, 126 bp, synthetic construct
  source 1..126: mol_type = other DNA
aagcgaggtcggaagaagcttttgtatatctttaaacagccctttatgaggcccgtacaaaccacacaagaggaggatgggtgctcatgcagatttcctgaagaggaagagggcggttgcgaactt

SEQ ID NO: 36 - protein, 112 aa, synthetic construct
RVKFSRSADAPAYKQGQNQLYNELNLGRREEYDVLDKRRGRDPEMGGKPRRKNPQEGLYNELQKDKMAEAYSEIGMKGERRRGKGHDGLYQGLSTATKDTYDALHMQALPPR

SEQ ID NO: 37 - DNA, 339 bp, synthetic construct
  source 1..339: mol_type = other DNA
agagtcaaattcagccgctccgcagatgcacctgcttataaacagggtcagaatcaattgtataatgaacttaatctcgggaggcgcgaggagtatgatgtgctggacaagcgacggggtcgagacccagagatgggcggtaaaccccgccgaaagaacccccaggagggactgtataatgagctgcaaaaggacaaaatggcagaagcctattccgaaatagggatgaagggagagcggcggcgaggtaagggacatgacggtctttatcaaggtcttagtactgcaactaaggacacctatgacgcgctgcatatgcaggctctcccacctagataa

SEQ ID NO: 38 - protein, 368 aa, synthetic construct
MALPVTALLLPLALLLHAARPQVQLVESGGGLVQPGGSLRLSCAASGFTFSSKTMGWARQVPGKAIEWLSGIYSDGSTYYADSVKGRFTISRDNAKNMVYLQMNSLKPEDTAVYYCATEDLTSYGRGTQVTVSSAAADYKDDDDKTTTPAPRPPTPAPTIASQPLSLRPEACRPAAGGAVHTRGLDFACDIYIWAPLAGTCGVLLLSLVITLYCKRGRKKLLYIFKQPFMRPVQTTQEEDGCSCRFPEEEEGGCELRVKFSRSADAPAYKQGQNQLYNELNLGRREEYDVLDKRRGRDPEMGGKPRRKNPQEGLYNELQKDKMAEAYSEIGMKGERRRGKGHDGLYQGLSTATKDTYDALHMQALPPR

SEQ ID NO: 39 - DNA, 1104 bp, synthetic construct
  source 1..1104: mol_type = other DNA
atggccttaccagtgaccgccttgctcctgccgctggccttgctgctccacgccgccaggccgcaagtgcaactggtggagtccggcgggggcctggtgcaacccggcggctccctgagactgagctgcgccgctagcggcttcaccttcagcagcaagaccatgggctgggctagacaagtgcccggcaaggccatcgagtggctgagcggcatctacagcgacggcagcacctactacgccgacagcgtgaagggcagattcaccatcagcagagacaacgccaagaacatggtgtacctgcagatgaacagcctgaagcccgaggacaccgccgtgtactactgcgccaccgaggacctgacaagctacggcagaggcacccaagtgaccgtgagcagcgccgctgccgactacaaggacgacgacgacaagacaacgacaccagcaccacggccacccactcctgctccgacaattgcgtctcagcccctttcccttcgacccgaagcttgtcgccctgctgcgggaggagcggtccacacgcgcgggcttgacttcgcttgcgacatctacatttgggcacccttggccgggacatgcggcgtcttgctcctgagtctggttataacgctgtattgtaagcgaggtcggaagaagcttttgtatatctttaaacagccctttatgaggcccgtacaaaccacacaagaggaggatgggtgctcatgcagatttcctgaagaggaagagggcggttgcgaacttagagtcaaattcagccgctccgcagatgcacctgcttataaacagggtcagaatcaattgtataatgaacttaatctcgggaggcgcgaggagtatgatgtgctggacaagcgacggggtcgagacccagagatgggcggtaaaccccgccgaaagaacccccaggagggactgtataatgagctgcaaaaggacaaaatggcagaagcctattccgaaatagggatgaagggagagcggcggcgaggtaagggacatgacggtctttatcaaggtcttagtactgcaactaaggacacctatgacgcgctgcatatgcaggctctcccacctaga

SEQ ID NO: 40 - protein, 373 aa, synthetic construct
MALPVTALLLPLALLLHAARPQVQLVESGGGLVQPGGSLRLSCAASGFTFSSYAMGWARQVPGKEVEWVSGIYSDGSTYYANSVKGRFTISRDNAKNTMYLQMNSLKPEDTAVYHCATDPTVHSDLPVWGQGTLVTVSSAAADYKDDDDKTTTPAPRPPTPAPTIASQPLSLRPEACRPAAGGAVHTRGLDFACDIYIWAPLAGTCGVLLLSLVITLYCKRGRKKLLYIFKQPFMRPVQTTQEEDGCSCRFPEEEEGGCELRVKFSRSADAPAYKQGQNQLYNELNLGRREEYDVLDKRRGRDPEMGGKPRRKNPQEGLYNELQKDKMAEAYSEIGMKGERRRGKGHDGLYQGLSTATKDTYDALHMQALPPR

SEQ ID NO: 41 - DNA, 1119 bp, synthetic construct
  source 1..1119: mol_type = other DNA
atggccttaccagtgaccgccttgctcctgccgctggccttgctgctccacgccgccaggccgcaagtgcaactcgtggagagcgggggggggctggtgcagcccggggggagcctgagactgagctgcgccgctagcggcttcaccttcagcagctacgccatgggctgggctagacaagtgcccggcaaagaggtggagtgggtgagcggcatctacagcgacggcagcacctactacgccaacagcgtgaagggcagattcaccatcagcagagacaacgccaagaacaccatgtacctgcagatgaacagcctgaagcccgaggacaccgccgtgtaccactgcgccacagatcccacagtgcacagcgatctgcccgtctgggggcaaggcaccctggtcaccgtgagcagcgccgctgccgactacaaggacgacgacgacaagacaacgacaccagcaccacggccacccactcctgctccgacaattgcgtctcagcccctttcccttcgacccgaagcttgtcgccctgctgcgggaggagcggtccacacgcgcgggcttgacttcgcttgcgacatctacatttgggcacccttggccgggacatgcggcgtcttgctcctgagtctggttataacgctgtattgtaagcgaggtcggaagaagcttttgtatatctttaaacagccctttatgaggcccgtacaaaccacacaagaggaggatgggtgctcatgcagatttcctgaagaggaagagggcggttgcgaacttagagtcaaattcagccgctccgcagatgcacctgcttataaacagggtcagaatcaattgtataatgaacttaatctcgggaggcgcgaggagtatgatgtgctggacaagcgacggggtcgagacccagagatgggcggtaaaccccgccgaaagaacccccaggagggactgtataatgagctgcaaaaggacaaaatggcagaagcctattccgaaatagggatgaagggagagcggcggcgaggtaagggacatgacggtctttatcaaggtcttagtactgcaactaaggacacctatgacgcgctgcatatgcaggctctcccacctaga

SEQ ID NO: 42 - protein, 372 aa, synthetic construct
MALPVTALLLPLALLLHAARPQVQLVESGGGLVQPGGSLRLSCAASGFTFSSYAMGWARQVPGKEVEWVSGIYSDGRTYYADSVKGRFTISRDNAKNEVYLQMNSLKPEDTAVYYCAPEPGQGVGDYWGQGTQVTVSSAAADYKDDDDKTTTPAPRPPTPAPTIASQPLSLRPEACRPAAGGAVHTRGLDFACDIYIWAPLAGTCGVLLLSLVITLYCKRGRKKLLYIFKQPFMRPVQTTQEEDGCSCRFPEEEEGGCELRVKFSRSADAPAYKQGQNQLYNELNLGRREEYDVLDKRRGRDPEMGGKPRRKNPQEGLYNELQKDKMAEAYSEIGMKGERRRGKGHDGLYQGLSTATKDTYDALHMQALPPR

SEQ ID NO: 43 - DNA, 1116 bp, synthetic construct
  source 1..1116: mol_type = other DNA
atggccttaccagtgaccgccttgctcctgccgctggccttgctgctccacgccgccaggccgcaagtgcagctcgtcgaaagcggcgggggcctggtgcaacctggcgggtccctgagactgagctgcgccgctagcggcttcaccttcagcagctacgccatgggctgggctagacaagtgcccggcaaagaggtggagtgggtgagcggcatctacagcgacggcagaacctactacgccgacagcgtgaagggcagattcaccatcagcagagacaacgccaagaacgaggtgtacctgcagatgaacagcctgaagcccgaggacaccgccgtctattactgtgcccccgagcctggccaaggcgtgggggattactggggccaaggcacccaagtgaccgtgagcagcgccgctgccgactacaaggacgacgacgacaagacaacgacaccagcaccacggccacccactcctgctccgacaattgcgtctcagcccctttcccttcgacccgaagcttgtcgccctgctgcgggaggagcggtccacacgcgcgggcttgacttcgcttgcgacatctacatttgggcacccttggccgggacatgcggcgtcttgctcctgagtctggttataacgctgtattgtaagcgaggtcggaagaagcttttgtatatctttaaacagccctttatgaggcccgtacaaaccacacaagaggaggatgggtgctcatgcagatttcctgaagaggaagagggcggttgcgaacttagagtcaaattcagccgctccgcagatgcacctgcttataaacagggtcagaatcaattgtataatgaacttaatctcgggaggcgcgaggagtatgatgtgctggacaagcgacggggtcgagacccagagatgggcggtaaaccccgccgaaagaacccccaggagggactgtataatgagctgcaaaaggacaaaatggcagaagcctattccgaaatagggatgaagggagagcggcggcgaggtaagggacatgacggtctttatcaaggtcttagtactgcaactaaggacacctatgacgcgctgcatatgcaggctctcccacctaga

SEQ ID NO: 44 - protein, 373 aa, synthetic construct
MALPVTALLLPLALLLHAARPQVQLVESGGGLVQPGGSLRLSCAASGFTFSSYAMGWARQVPGKDVEWVSGIYSDGSTNYADSVKGRFTISRDNAKNTVYLQMNSLRPEDTAVYHCATDPTVHSDLPVWGQGTLVTVSSAAADYKDDDDKTTTPAPRPPTPAPTIASQPLSLRPEACRPAAGGAVHTRGLDFACDIYIWAPLAGTCGVLLLSLVITLYCKRGRKKLLYIFKQPFMRPVQTTQEEDGCSCRFPEEEEGGCELRVKFSRSADAPAYKQGQNQLYNELNLGRREEYDVLDKRRGRDPEMGGKPRRKNPQEGLYNELQKDKMAEAYSEIGMKGERRRGKGHDGLYQGLSTATKDTYDALHMQALPPR

SEQ ID NO: 45 - DNA, 1119 bp, synthetic construct
  source 1..1119: mol_type = other DNA
atggccttaccagtgaccgccttgctcctgccgctggccttgctgctccacgccgccaggccgcaagtgcaactcgtggagagcgggggggggctggtgcagcccggggggagcctgagactgagctgcgccgctagcggcttcaccttcagcagctacgccatgggctgggctagacaagtgcccggcaaagacgtggagtgggtgagcggcatctacagcgacggcagcaccaactacgccgacagcgtgaagggcagattcaccatcagcagagacaacgccaagaacaccgtgtacctgcagatgaacagcctgagacccgaggacaccgccgtgtaccactgcgccacagatcccacagtgcacagcgatctgcccgtctgggggcaaggcaccctggtcaccgtgagcagcgccgctgccgactacaaggacgacgacgacaagacaacgacaccagcaccacggccacccactcctgctccgacaattgcgtctcagcccctttcccttcgacccgaagcttgtcgccctgctgcgggaggagcggtccacacgcgcgggcttgacttcgcttgcgacatctacatttgggcacccttggccgggacatgcggcgtcttgctcctgagtctggttataacgctgtattgtaagcgaggtcggaagaagcttttgtatatctttaaacagccctttatgaggcccgtacaaaccacacaagaggaggatgggtgctcatgcagatttcctgaagaggaagagggcggttgcgaacttagagtcaaattcagccgctccgcagatgcacctgcttataaacagggtcagaatcaattgtataatgaacttaatctcgggaggcgcgaggagtatgatgtgctggacaagcgacggggtcgagacccagagatgggcggtaaaccccgccgaaagaacccccaggagggactgtataatgagctgcaaaaggacaaaatggcagaagcctattccgaaatagggatgaagggagagcggcggcgaggtaagggacatgacggtctttatcaaggtcttagtactgcaactaaggacacctatgacgcgctgcatatgcaggctctcccacctaga

SEQ ID NO: 46 - protein, 372 aa, synthetic construct
MALPVTALLLPLALLLHAARPQVQLVESGGGLVQPGGSLRLSCAASGFTFSSYDMGWARQVPGKAVEWVSGIYSDGSTYYADSVKGRFTISRDNAKNTVYLQMNSLKPEDTAVYYCATDPLTSELRSWGQGTQVTVSSAAADYKDDDDKTTTPAPRPPTPAPTIASQPLSLRPEACRPAAGGAVHTRGLDFACDIYIWAPLAGTCGVLLLSLVITLYCKRGRKKLLYIFKQPFMRPVQTTQEEDGCSCRFPEEEEGGCELRVKFSRSADAPAYKQGQNQLYNELNLGRREEYDVLDKRRGRDPEMGGKPRRKNPQEGLYNELQKDKMAEAYSEIGMKGERRRGKGHDGLYQGLSTATKDTYDALHMQALPPR

SEQ ID NO: 47 - DNA, 1116 bp, synthetic construct
  source 1..1116: mol_type = other DNA
atggccttaccagtgaccgccttgctcctgccgctggccttgctgctccacgccgccaggccgcaagtgcagctggtcgaaagcggcggcgggctcgtgcagcccggcggcagcctgagactgagctgcgccgctagcggcttcaccttcagcagctacgacatgggctgggctagacaagtgcccggcaaggccgtggagtgggtgagcggcatctacagcgacggcagcacctactacgccgacagcgtgaagggcagattcaccatcagcagagacaacgccaagaacaccgtgtacctgcagatgaacagcctgaagcccgaggacaccgccgtgtactactgcgccaccgaccccctgacaagcgagctgagaagctggggccaaggcacccaagtgaccgtgagcagcgccgctgccgactacaaggacgacgacgacaagacaacgacaccagcaccacggccacccactcctgctccgacaattgcgtctcagcccctttcccttcgacccgaagcttgtcgccctgctgcgggaggagcggtccacacgcgcgggcttgacttcgcttgcgacatctacatttgggcacccttggccgggacatgcggcgtcttgctcctgagtctggttataacgctgtattgtaagcgaggtcggaagaagcttttgtatatctttaaacagccctttatgaggcccgtacaaaccacacaagaggaggatgggtgctcatgcagatttcctgaagaggaagagggcggttgcgaacttagagtcaaattcagccgctccgcagatgcacctgcttataaacagggtcagaatcaattgtataatgaacttaatctcgggaggcgcgaggagtatgatgtgctggacaagcgacggggtcgagacccagagatgggcggtaaaccccgccgaaagaacccccaggagggactgtataatgagctgcaaaaggacaaaatggcagaagcctattccgaaatagggatgaagggagagcggcggcgaggtaagggacatgacggtctttatcaaggtcttagtactgcaactaaggacacctatgacgcgctgcatatgcaggctctcccacctaga

SEQ ID NO: 48 - protein, 373 aa, synthetic construct
MALPVTALLLPLALLLHAARPQVQLVESGGGLVQPGGSLRLSCTASGFTFSSYAMGWARQVPGKEVEWVSGIYSDGSTNYADSVKGRFTISRDNAKNTVYLQMNSLRPEDTAVYHCATDPTVHSDLPVWGQGTLVTVSSAAADYKDDDDKTTTPAPRPPTPAPTIASQPLSLRPEACRPAAGGAVHTRGLDFACDIYIWAPLAGTCGVLLLSLVITLYCKRGRKKLLYIFKQPFMRPVQTTQEEDGCSCRFPEEEEGGCELRVKFSRSADAPAYKQGQNQLYNELNLGRREEYDVLDKRRGRDPEMGGKPRRKNPQEGLYNELQKDKMAEAYSEIGMKGERRRGKGHDGLYQGLSTATKDTYDALHMQALPPR

SEQ ID NO: 49 - DNA, 1119 bp, synthetic construct
  source 1..1119: mol_type = other DNA
atggccttaccagtgaccgccttgctcctgccgctggccttgctgctccacgccgccaggccgcaagtgcaactcgtggagagcgggggggggctggtgcagcccggggggagcctgagactgagctgcaccgctagcggcttcaccttcagcagctacgccatgggctgggctagacaagtgcccggcaaagaggtggagtgggtgagcggcatctacagcgacggcagcaccaactacgccgacagcgtgaagggcagattcaccatcagcagagacaacgccaagaacaccgtgtacctgcagatgaacagcctgagacccgaggacaccgccgtgtaccactgcgccacagatcccacagtgcacagcgatctgcccgtctgggggcaaggcaccctggtcaccgtgagcagcgccgctgccgactacaaggacgacgacgacaagacaacgacaccagcaccacggccacccactcctgctccgacaattgcgtctcagcccctttcccttcgacccgaagcttgtcgccctgctgcgggaggagcggtccacacgcgcgggcttgacttcgcttgcgacatctacatttgggcacccttggccgggacatgcggcgtcttgctcctgagtctggttataacgctgtattgtaagcgaggtcggaagaagcttttgtatatctttaaacagccctttatgaggcccgtacaaaccacacaagaggaggatgggtgctcatgcagatttcctgaagaggaagagggcggttgcgaacttagagtcaaattcagccgctccgcagatgcacctgcttataaacagggtcagaatcaattgtataatgaacttaatctcgggaggcgcgaggagtatgatgtgctggacaagcgacggggtcgagacccagagatgggcggtaaaccccgccgaaagaacccccaggagggactgtataatgagctgcaaaaggacaaaatggcagaagcctattccgaaatagggatgaagggagagcggcggcgaggtaagggacatgacggtctttatcaaggtcttagtactgcaactaaggacacctatgacgcgctgcatatgcaggctctcccacctaga

SEQ ID NO: 50 - protein, 373 aa, synthetic construct
MALPVTALLLPLALLLHAARPQVQLVESGGGLVQPGGSLRLSCAASGFTFSSYAMGWARQVPGKEVEWVSGIYSDGSTNYADSVKGRFTISRDNAKNTVYLQMNSLRPEDTAVYHCATDPTVHSDLPVWGQGTLVTVSSAAADYKDDDDKTTTPAPRPPTPAPTIASQPLSLRPEACRPAAGGAVHTRGLDFACDIYIWAPLAGTCGVLLLSLVITLYCKRGRKKLLYIFKQPFMRPVQTTQEEDGCSCRFPEEEEGGCELRVKFSRSADAPAYKQGQNQLYNELNLGRREEYDVLDKRRGRDPEMGGKPRRKNPQEGLYNELQKDKMAEAYSEIGMKGERRRGKGHDGLYQGLSTATKDTYDALHMQALPPR

SEQ ID NO: 51 - DNA, 1119 bp, synthetic construct
  source 1..1119: mol_type = other DNA
atggccttaccagtgaccgccttgctcctgccgctggccttgctgctccacgccgccaggccgcaagtgcaactcgtggagagcgggggggggctggtgcagcccggggggagcctgagactgagctgcgccgctagcggcttcaccttcagcagctacgccatgggctgggctagacaagtgcccggcaaagaggtggagtgggtgagcggcatctacagcgacggcagcaccaactacgccgacagcgtgaagggcagattcaccatcagcagagacaacgccaagaacaccgtgtacctgcagatgaacagcctgagacccgaggacaccgccgtgtaccactgcgccacagatcccacagtgcacagcgatctgcccgtctgggggcaaggcaccctggtcaccgtgagcagcgccgctgccgactacaaggacgacgacgacaagacaacgacaccagcaccacggccacccactcctgctccgacaattgcgtctcagcccctttcccttcgacccgaagcttgtcgccctgctgcgggaggagcggtccacacgcgcgggcttgacttcgcttgcgacatctacatttgggcacccttggccgggacatgcggcgtcttgctcctgagtctggttataacgctgtattgtaagcgaggtcggaagaagcttttgtatatctttaaacagccctttatgaggcccgtacaaaccacacaagaggaggatgggtgctcatgcagatttcctgaagaggaagagggcggttgcgaacttagagtcaaattcagccgctccgcagatgcacctgcttataaacagggtcagaatcaattgtataatgaacttaatctcgggaggcgcgaggagtatgatgtgctggacaagcgacggggtcgagacccagagatgggcggtaaaccccgccgaaagaacccccaggagggactgtataatgagctgcaaaaggacaaaatggcagaagcctattccgaaatagggatgaagggagagcggcggcgaggtaagggacatgacggtctttatcaaggtcttagtactgcaactaaggacacctatgacgcgctgcatatgcaggctctcccacctaga

SEQ ID NO: 52 - protein, 373 aa, synthetic construct
MALPVTALLLPLALLLHAARPQVQLVESGGGLVQPGGSLRLSCAASGFTFSSYAMGWARQVPGKEVEWVSGIYSDGSTNYADSVKGRFTISRDNAKNTVYLQMNSLRPEDTAVYHCATDPTVHSDLPVWGQGTQVTVSSAAADYKDDDDKTTTPAPRPPTPAPTIASQPLSLRPEACRPAAGGAVHTRGLDFACDIYIWAPLAGTCGVLLLSLVITLYCKRGRKKLLYIFKQPFMRPVQTTQEEDGCSCRFPEEEEGGCELRVKFSRSADAPAYKQGQNQLYNELNLGRREEYDVLDKRRGRDPEMGGKPRRKNPQEGLYNELQKDKMAEAYSEIGMKGERRRGKGHDGLYQGLSTATKDTYDALHMQALPPR

SEQ ID NO: 53 - DNA, 1119 bp, synthetic construct
  source 1..1119: mol_type = other DNA
atggccttaccagtgaccgccttgctcctgccgctggccttgctgctccacgccgccaggccgcaagtgcaactcgtggagagcgggggggggctggtgcagcccggggggagcctgagactgagctgcgccgctagcggcttcaccttcagcagctacgccatgggctgggctagacaagtgcccggcaaagaggtggagtgggtgagcggcatctacagcgacggcagcaccaactacgccgacagcgtgaagggcagattcaccatcagcagagacaacgccaagaacaccgtgtacctgcagatgaacagcctgagacccgaggacaccgccgtgtaccactgcgccacagatcccacagtgcacagcgatctgcccgtctgggggcaaggcacccaagtcaccgtgagcagcgccgctgccgactacaaggacgacgacgacaagacaacgacaccagcaccacggccacccactcctgctccgacaattgcgtctcagcccctttcccttcgacccgaagcttgtcgccctgctgcgggaggagcggtccacacgcgcgggcttgacttcgcttgcgacatctacatttgggcacccttggccgggacatgcggcgtcttgctcctgagtctggttataacgctgtattgtaagcgaggtcggaagaagcttttgtatatctttaaacagccctttatgaggcccgtacaaaccacacaagaggaggatgggtgctcatgcagatttcctgaagaggaagagggcggttgcgaacttagagtcaaattcagccgctccgcagatgcacctgcttataaacagggtcagaatcaattgtataatgaacttaatctcgggaggcgcgaggagtatgatgtgctggacaagcgacggggtcgagacccagagatgggcggtaaaccccgccgaaagaacccccaggagggactgtataatgagctgcaaaaggacaaaatggcagaagcctattccgaaatagggatgaagggagagcggcggcgaggtaagggacatgacggtctttatcaaggtcttagtactgcaactaaggacacctatgacgcgctgcatatgcaggctctcccacctaga

SEQ ID NO: 54 - protein, 373 aa, synthetic construct
MALPVTALLLPLALLLHAARPQVQLVESGGGLVQPGGSLRLSCAASGFTFSSYAMGWARQVPGKDVEWVSGIYSDGSTYYADSVKGRFTISRYNAKNTVYLQMNSLKPEDTAVYYCATDPTLENQTTAWGQGTQVTVSSAAADYKDDDDKTTTPAPRPPTPAPTIASQPLSLRPEACRPAAGGAVHTRGLDFACDIYIWAPLAGTCGVLLLSLVITLYCKRGRKKLLYIFKQPFMRPVQTTQEEDGCSCRFPEEEEGGCELRVKFSRSADAPAYKQGQNQLYNELNLGRREEYDVLDKRRGRDPEMGGKPRRKNPQEGLYNELQKDKMAEAYSEIGMKGERRRGKGHDGLYQGLSTATKDTYDALHMQALPPR

SEQ ID NO: 55 - DNA, 1119 bp, synthetic construct
  source 1..1119: mol_type = other DNA
atggccttaccagtgaccgccttgctcctgccgctggccttgctgctccacgccgccaggccgcaagtgcagctggtcgagagcggcgggggcctcgtccaacccggcggcagcctgagactgagctgcgccgctagcggcttcaccttcagcagctacgccatgggctgggctagacaagtgcccggcaaggacgtggagtgggtgagcggcatctacagcgacggcagcacctactacgccgacagcgtgaagggcagattcaccatcagcagatacaacgccaagaacaccgtgtacctgcagatgaacagcctgaagcccgaggacaccgccgtgtactactgcgccaccgatcctaccctcgagaatcagacaaccgcctggggccaagggacccaagtgaccgtgagcagcgccgctgccgactacaaggacgacgacgacaagacaacgacaccagcaccacggccacccactcctgctccgacaattgcgtctcagcccctttcccttcgacccgaagcttgtcgccctgctgcgggaggagcggtccacacgcgcgggcttgacttcgcttgcgacatctacatttgggcacccttggccgggacatgcggcgtcttgctcctgagtctggttataacgctgtattgtaagcgaggtcggaagaagcttttgtatatctttaaacagccctttatgaggcccgtacaaaccacacaagaggaggatgggtgctcatgcagatttcctgaagaggaagagggcggttgcgaacttagagtcaaattcagccgctccgcagatgcacctgcttataaacagggtcagaatcaattgtataatgaacttaatctcgggaggcgcgaggagtatgatgtgctggacaagcgacggggtcgagacccagagatgggcggtaaaccccgccgaaagaacccccaggagggactgtataatgagctgcaaaaggacaaaatggcagaagcctattccgaaatagggatgaagggagagcggcggcgaggtaagggacatgacggtctttatcaaggtcttagtactgcaactaaggacacctatgacgcgctgcatatgcaggctctcccacctaga

SEQ ID NO: 56 - protein, 373 aa, synthetic construct
MALPVTALLLPLALLLHAARPQVQLVESGGGLVQPGGSLRLACAASGFTFSSYAMGWARQVPGKDVEWVSGIYSDGSTYYADSVKGRFTISRDNAKNTVYLQMNSLKPEDTAVYYCATDPTLENQTTAWGQGTQVTVSSAAADYKDDDDKTTTPAPRPPTPAPTIASQPLSLRPEACRPAAGGAVHTRGLDFACDIYIWAPLAGTCGVLLLSLVITLYCKRGRKKLLYIFKQPFMRPVQTTQEEDGCSCRFPEEEEGGCELRVKFSRSADAPAYKQGQNQLYNELNLGRREEYDVLDKRRGRDPEMGGKPRRKNPQEGLYNELQKDKMAEAYSEIGMKGERRRGKGHDGLYQGLSTATKDTYDALHMQALPPR

SEQ ID NO: 57 - DNA, 1119 bp, synthetic construct
  source 1..1119: mol_type = other DNA
atggccttaccagtgaccgccttgctcctgccgctggccttgctgctccacgccgccaggccgcaagtgcaactggtcgaaagcgggggcggcctggtgcagcccggcggcagcctgagactggcctgcgccgctagcggcttcaccttcagcagctacgccatgggctgggctagacaagtgcccggcaaggacgtggagtgggtgagcggcatctacagcgacggcagcacctactacgccgacagcgtgaagggcagattcaccatcagcagagacaacgccaagaacaccgtgtacctgcagatgaacagcctgaagcccgaggacaccgccgtgtactactgcgccacagatcccacactggagaaccaaaccaccgcttgggggcaaggcacccaagtgaccgtgagcagcgccgctgccgactacaaggacgacgacgacaagacaacgacaccagcaccacggccacccactcctgctccgacaattgcgtctcagcccctttcccttcgacccgaagcttgtcgccctgctgcgggaggagcggtccacacgcgcgggcttgacttcgcttgcgacatctacatttgggcacccttggccgggacatgcggcgtcttgctcctgagtctggttataacgctgtattgtaagcgaggtcggaagaagcttttgtatatctttaaacagccctttatgaggcccgtacaaaccacacaagaggaggatgggtgctcatgcagatttcctgaagaggaagagggcggttgcgaacttagagtcaaattcagccgctccgcagatgcacctgcttataaacagggtcagaatcaattgtataatgaacttaatctcgggaggcgcgaggagtatgatgtgctggacaagcgacggggtcgagacccagagatgggcggtaaaccccgccgaaagaacccccaggagggactgtataatgagctgcaaaaggacaaaatggcagaagcctattccgaaatagggatgaagggagagcggcggcgaggtaagggacatgacggtctttatcaaggtcttagtactgcaactaaggacacctatgacgcgctgcatatgcaggctctcccacctaga

SEQ ID NO: 58 - protein, 498 aa, synthetic construct
MALPVTALLLPLALLLHAARPEVQLQQSGPELVKPGASVKMSCKASGYTFTSYFIHWVKQKPGQGLEWIGFINPYNDGSKYNEKFKGKATLTSDKSSSTAYMELSSLTSEDSAVYYCTRDDGYYGYAMDYWGQGTSVTVSSGGGGSGGGGSGGGGSDIQMTQSPSSLSASLGERVSLTCRATQELSGYLSWLQQKPDGTIKRLIYAASTLDSGVPKRFSGNRSGSDYSLTISSLESEDFADYYCLQYAIYPYTFGGGTKLEIKRAAADYKDDDDKTTTPAPRPPTPAPTIASQPLSLRPEACRPAAGGAVHTRGLDFACDIYIWAPLAGTCGVLLLSLVITLYCKRGRKKLLYIFKQPFMRPVQTTQEEDGCSCRFPEEEEGGCELRVKFSRSADAPAYKQGQNQLYNELNLGRREEYDVLDKRRGRDPEMGGKPRRKNPQEGLYNELQKDKMAEAYSEIGMKGERRRGKGHDGLYQGLSTATKDTYDALHMQALPPR

SEQ ID NO: 59 - DNA, 1494 bp, synthetic construct
  source 1..1494: mol_type = other DNA
atggccttaccagtgaccgccttgctcctgccgctggccttgctgctccacgccgccaggccggaggtgcagctgcagcagagcggccccgagctggtgaagcccggcgctagcgtgaagatgagctgcaaggctagcggctacaccttcacaagctacttcatccactgggtgaaacagaagcccggccaaggcctggagtggatcggcttcatcaacccctacaacgacggcagcaagtacaacgagaagttcaagggcaaggccaccctcacaagcgacaagagcagcagcaccgcctacatggagctgagcagcctgacaagcgaagacagcgccgtgtactactgcacaagagacgacggctactacggctacgccatggactactggggccaaggcacaagcgtcaccgtgagcagcgggggcgggggcagcggcgggggggggagcggcgggggcggcagcgacattcagatgacacagagccctagcagcctgagcgctagcctgggcgagagagtgagcctgacctgcagagccacccaagagctgagcggctacctgagctggctgcagcagaagcctgacggcaccatcaagagactgatctacgccgctagcaccctggacagcggcgtgcccaagagattcagcggcaacagaagcggcagcgactacagcctgaccatcagcagcctggagagcgaggacttcgccgactactactgcctgcagtacgccatctacccctacaccttcggcgggggcaccaagctggagatcaagagagccgctgccgactacaaggacgacgacgacaagacaacgacaccagcaccacggccacccactcctgctccgacaattgcgtctcagcccctttcccttcgacccgaagcttgtcgccctgctgcgggaggagcggtccacacgcgcgggcttgacttcgcttgcgacatctacatttgggcacccttggccgggacatgcggcgtcttgctcctgagtctggttataacgctgtattgtaagcgaggtcggaagaagcttttgtatatctttaaacagccctttatgaggcccgtacaaaccacacaagaggaggatgggtgctcatgcagatttcctgaagaggaagagggcggttgcgaacttagagtcaaattcagccgctccgcagatgcacctgcttataaacagggtcagaatcaattgtataatgaacttaatctcgggaggcgcgaggagtatgatgtgctggacaagcgacggggtcgagacccagagatgggcggtaaaccccgccgaaagaacccccaggagggactgtataatgagctgcaaaaggacaaaatggcagaagcctattccgaaatagggatgaagggagagcggcggcgaggtaagggacatgacggtctttatcaaggtcttagtactgcaactaaggacacctatgacgcgctgcatatgcaggctctcccacctaga